European Patent Specification EP 4 356 137 B1, published July 23, 2025. Title: Collagen Type XX Assay. Applicant: Nordic Bioscience A/S. The sequence listing filed with the application follows.

SEQUENCE LISTING (21 sequences)

SEQ ID NO: 1 - protein, 10 aa, Artificial Sequence
  Synthetic peptide
QGASTQGLWE

SEQ ID NO: 2 - protein, 11 aa, Artificial Sequence
  Synthetic Peptide
QGASTQGLWES

SEQ ID NO: 3 - protein, 8 aa, Artificial Sequence
  Synthetic Peptide
QGASTQGL

SEQ ID NO: 4 - protein, 10 aa, Artificial Sequence
  MOD_RES 1: Amino acid is biotinylated via an optional linker
  Synthetic peptide
QGASTQGLWE

SEQ ID NO: 5 - protein, 10 aa, Artificial Sequence
  MOD_RES 1: Biotinylated
  Synthetic peptide
QGASTQGLWE

SEQ ID NO: 6 - protein, 30 aa, Artificial Sequence
  Synthetic peptide
RHLEGRGEPGAVGQMGSPGQQGASTQGLWE

SEQ ID NO: 7 - protein, 13 aa, Artificial Sequence
  MOD_RES 1: Bound to keyhole limpet hemocyanin
  Synthetic peptide
CGGQGASTQGLWE

SEQ ID NO: 8 - protein, 10 aa, Artificial Sequence
  Synthetic peptide
SHAHQRTGGN

SEQ ID NO: 9 - protein, 10 aa, Artificial Sequence
  MOD_RES 1: Biotinylated
  Synthetic peptide
SHAHQRTGGN

SEQ ID NO: 10 - protein, 13 aa, Artificial Sequence
  Synthetic peptide
  MOD_RES 13: Bound to keyhole limpet hemocyanin
IRQCPDRTYGGGC

SEQ ID NO: 11 - protein, 5 aa, Artificial Sequence
  CDR
DYSMH

SEQ ID NO: 12 - protein, 17 aa, Artificial Sequence
  CDR
WINTETGEPTYADGFKG

SEQ ID NO: 13 - protein, 16 aa, Artificial Sequence
  CDR
RSSQSIVHNNGKIYLE

SEQ ID NO: 14 - protein, 7 aa, Artificial Sequence
  CDR
KVSNRFS

SEQ ID NO: 15 - protein, 9 aa, Artificial Sequence
  CDR
FQGSHVPYT

SEQ ID NO: 16 - protein, 79 aa, Artificial Sequence
  light chain variable region
RSSQSIVHNNGKIYLEWFLQKPGQSPKALIQKVSNRFSGVPDRFSGSGSGTDFTLKISRVEAEDLGVYYCFQGSHVPYT

SEQ ID NO: 17 - protein, 71 aa, Artificial Sequence
  heavy chain variable region
DYSMHWVKQAPGKGLKWMGWINTETGEPTYADGFKGRFAFSLETSASTAYLKINNLKNDDTATYFCARGPY

SEQ ID NO: 18 - protein, 112 aa, Artificial Sequence
  light chain variable region
DVLLTQTPLSLPVSLGDQASISCRSSQSIVHNNGKIYLEWFLQKPGQSPKALIQKVSNRFSGVPDRFSGSGSGTDFTLKISRVEAEDLGVYYCFQGSHVPYTFGGGTKLEIK

SEQ ID NO: 19 - protein, 112 aa, Artificial Sequence
  heavy chain variable region
QIQLMQSGPELKKPGETVKISCKASGYPFTDYSMHWVKQAPGKGLKWMGWINTETGEPTYADGFKGRFAFSLETSASTAYLKINNLKNDDTATYFCARGPYWGQGTLVTVSA

SEQ ID NO: 20 - protein, 511 aa, Artificial Sequence
  antibody heavy chain
QIQLMQSGPELKKPGETVKISCKASGYPFTDYSMHWVKQAPGKGLKWMGWINTETGEPTYADGFKGRFAFSLETSASTAYLKINNLKNDDTATYFCARGPYWGQGTLVTVSAAKTTAPSVYPLAPVCGDTTGSSVTLGCLVKGYFPEPVTLTWNSGSLSSGVHTFPAVLQSDLYTLSSSVTVTSSTWPSQSITCNVAHPASSTKVDKKIEPRGPTIKPCPPCKCPAPNLLGGPSVFIFPPKIKDVLMISLSPIVTCVVVDVSEDDPDVQISWFVNNVEVHTAQTQTHREDYNSTLRVVSALPIQHQDWMSGKEFKCKVNNKDLPAPIERTISKPKGSVRAPQVYVLPPPEEEMTKKQVTLTCMVTDFMPEDIYVEWTNNGKTELNYKNTEPVLDSDGSYFMYSKLRVEKKNWVERNSYSCSVVHEGLHNHHTTKSFSRTPGLDLDDVCAEAQDGELDGLWTTITIFISLFLLSVCYSASVTLFKVKWIFSSVVELKQTISPDYRNMIGQGA

SEQ ID NO: 21 - protein, 219 aa, Artificial Sequence
  antibody light chain
DVLLTQTPLSLPVSLGDQASISCRSSQSIVHNNGKIYLEWFLQKPGQSPKALIQKVSNRFSGVPDRFSGSGSGTDFTLKISRVEAEDLGVYYCFQGSHVPYTFGGGTKLEIKRADAAPTVSIFPPSSEQLTSGGASVVCFLNNFYPKDINVKWKIDGSERQNGVLNSWTDQDSKDSTYSMSSTLTLTKDEYERHNSYTCEATHKTSTSPIVKSFNRNEC